European Patent Specification EP 4 050 094 B1, published February 21, 2024. Title: HIGH-EFFICIENCY PETROLEUM DEGRADING BACTERIUM TDYN1T AND USE THEREOF. Applicant: TIANJIN UNIVERSITY; TIANJIN JC ENVIRONMENTAL SERVICES. The sequence listing filed with the application follows.

SEQUENCE LISTING (1 sequence)

SEQ ID NO: 1 - DNA, 1357 bp, None(Falsochrobactrum sp)
tgcagtcgacgagcccttcggggttagtggcagacgggtgagtaatgcatgggaatctaccgttctctacggaataactcagggaaacttgtgctaataccgtatacgcccttttggggaaagatttatcggggaacgatgagcccatgttggattagctagttggtggggtaaaggcccaccaaggcgacgatccatagctggtctgagaggatgatcagccacactgggactgagacacggcccagactcctacgggaggcagcagtggggaatattggacaatgggcgcaagcctgatccagccatgccgcgtgagtgatgaaggccttagggttgtaaagctctttcaccggtgaagataatgacggtaaccggagaagaagccccggctaacttcgtgccagcagccgcggtaatacgaagggggctagcgttgttcggaattactgggcgtaaagcgcgcgtaggcggattggtcagttaggggtgaaatcccagggctcaaccctggaactgcctttaatactgccagtcttgagtatggaagaggtgagtggaattccgagtgtagaggtgaaattcgtagatattcggaggaacaccagtggcgaatgcggctcactggtccattactgacgctgaggtgcgaaagcgtgatgagcaaacaggattagataccctggtagtccacgccgtaaactatgaatgttagccgtcggggggtttacctttcggtggcgcagctaacgcattaaacattccgcctggggagtacggtcgcaagattaaaactcaaaggaattgacgggggcccgcacaagcggtggagcatgtggtttaattcgaagcaacgcgcagaaccttaccagcccttgacataccggtcgcggatcgagagatcgatctttcagttcggctggaccggatacaggtgctgcatggctgtcgtcagctcgtgtcgtgagatgttgggttaagtcccgcaacgagcgcaaccctcgcccttagttgccagcattcagttgggcactctaaggggactgccggtgataagccgagaggaaggtggggatgacgtcaagtcctcatggcccttacgggctgggctacacacgtgctacaatggtggtgacagtgggcagcgagcacgcgagtgtgagctaatctccaaaaaccatctcagttcggattgcactctgcaactcgagtgcatgaagttggaatcgctagtaatcgcggatcagcatgccgcggtgaatacgttcccgggccttgtacacaccgcccgtcacaccatgggagttggttttacctagaaggcgctgtgctaaccgcaaggaggcaggcgaccacg